European Patent Specification EP 3 704 238 B1, published January 3, 2024. Title: ENGINEERED NUCLEASES THAT TARGET HUMAN AND CANINE FACTOR VIII GENES AS A TREATMENT FOR HEMOPHILIA A. Applicant: Hekele, Armin Beard, Clayton Jantz, Derek Smith, James J Bartsevich, Victor. The sequence listing filed with the application follows.

SEQUENCE LISTING (50 sequences)

SEQ ID NO: 1 - protein, 163 aa, Chlamydomonas reinhardtii
MNTKYNKEFLLYLAGFVDGDGSIIAQIKPNQSYKFKHQLSLAFQVTQKTQRRWFLDKLVDEIGVGYVRDRGSVSDYILSEIKPLHNFLTQLQPFLKLKQKQANLVLKIIWRLPSAKESPDKFLEVCTWVDQIAALNDSKTRKTTSETVRAVLDSLSEKKKSSP

SEQ ID NO: 2 - protein, 9 aa, Chlamydomonas reinhardtii
LAGLIDADG

SEQ ID NO: 3 - DNA, 9512 bp, Homo sapiens
ttgaacagtcactgagcaactactatgtcctgggttctaattcaggggtgggcaaactatagccccagaatttggcccatagcctgcttttgtacggactgtgagttaagaatagtttttacacgttgaaaggattgcaaagacaaacatacaaagaaacaaagaagactgtgcaacagagaccacctgtggtctgtaaagactaacacatttctatcccgcccttgacagaaagagtctgtgggctgctggtctcctctaacggtggtagagatgcctgcacggttaacattaatccttggcaccagaatcctcagcacctaggaaccagatcttgcctaacacgctaatttcagtcttgaccaccttcctccggcgtagcggttctcaaacgtctttgtctttgtactattcacgtataaaatattctttcataagcaacatttatccttttgggaatacctcacaatggggagaaggggaaccccaacagcctttaagggttcactgcttcgctgccaccatttccgacggtttacactgttttaagtgtgaatttggaattgttttcaagttaaaaagcaaactaatcatgtcctctgaaagtatttgcttttggcatgctagaaatcagtgttgacttttgatactgatgtgatacattacgagggaattctcaaaactgctgaaatctggcctcggcccagttatcactgctcttaagcttctgagggagatacatgaatgagcccacggcaaatggaaaacgaggagttttagtgtttcctagaattatgctcagatacccactacctgaccgtctggttatccttcccctcacctccctgacgcaaggagtttggaccagaggcctaaggaggcttctcctgaagcccaaatcccaaactggtcaccagtcatgctccgtaactcctgaacctgacaagaagccagccggccaggtctgcagcccgggttaagaggagcataccaggaaagagccaaagagcaaaggagcatgagcccttcaaccgcttttacaataatttgggctaggcgttcagggctccgtaggacccttcctggcagccaagtgagagaaagaggaatgatggtggaatgggcctctcctgtgcttcccattacttccacactgtcgaaatagaaatagaagcagaaaagaacaccctacaagtcccacccatttggaggcactcaactcacagtgacaaccctccacacctctcccctgcaaaaagacgcaaaacaaaaacacctactccaaactgtgtccttacatctcagccccgaagatcaggattgtgtgcaacttcggcccaaaggatgcatttccccagggttgaaagtttgagaaagaggctatattctgaagagttcttgttgtcaccatcaaaaggattaaaaagacgcaataaataagaaaacagcgtagttggggggcatgctccatttgagccagaaagccttggaaacttaagtgttctcaaacggaacgccatcctgctttgggggaacacggaggctgccttgcagtcacgtgatcgcacaacaccaaagggccacgcactctgatttcacctacttaactaaaagttgcagcaaaatccctattacaggccaggcgtggtggctcatgcctgtaatcccagcactttgggaggccgaggagggtggatcatttgaggtcaggagttggagaccagcttggccaacatggtgagaccccatctctattaaaaatacaaaaattagcccagcgtggtggtgcacgcctgtaatcccaggcaccctggaggttgaggtaggagaatcgcttgaacccaggaggcggaggttgcagtgagccgagatcacgccactgcgctcctgcctgggcgacagagtgagactccatctcggggaaaaaaaaaaaaaaaaaaaaaaaaatccctattacaaataaaagctgttgtgatccagactgcatatacctctgcgaatggaaccagaaccgtgaattccaatgcaaatcgatgcatcggcaccagacccgctgcactggatgtatctgcattgcagtcacccgagtacggagcacatcatagatgatctctgcaggttcgttgcccacataggaggcatagcgcaaatttcaaaggaacgaatacatcctggagcccaaacagctatctggttctgctgctggcctcctgacaagtaggtaagagagtcacattttatagacgacggacaccaaaaccacacatgaggagtacaagagtagctttatcatggatttagggctgtggttacaaggaagctgtaaggaataaaatgactcccatgaagacgtaccgtgcggacgagtggaaggagaaatttggccattacaaagacacaggaatatgttaagaagtgaggggcaggatgaaatcatctagggtaggtatttagagggagggcgccgtgcaaaataaaatcctcactatgaaacaaaggcggaggcaggaggctgcgttaggtggaagcagcggaggaaggagacgaaagggattgtcattttcatgtcgtggctttttagaagacagccatgtcctctactctgattctatcaaaatgtgttctcggggtgctggtaacgttcagccaacgaaataattcctatggcggcagtaggaataacaaaacgcagaagcgggaacgatgtctttttattcctccccagacgcaaacgtggatgcatgaggtttggtaacaggcaaagtcatctggttaacgtgactgatgcaaaaagtccaggcctgggcaaaaagaagtcactgggtgaatgggatggatcagactccctgtcctgagggggagatggtttcttgcagaacgaggtgaaggaggtggttctgctcagcagtcaacagtggccacatctccacctgcagcgacttgatggcttccgtgtccttttcgtgggtagccatgaccaaagactggagcagcagaaagagctcctcgggaagctggccgctgctctcctgcccgtggctgtcaaaagcctcccaggagtacttctccagggtctgggcgtgctccggcagcagcttggcgggcggtggttgcaggaggagcagcagcagcacgcgggacacctcgcagcggaccagcacgtccgagaaggcgcccagggcggcgggagagggcgccgccgagccggagttcggaggaagcagcgcggccggtagggcgggcgtcgccccgggcccgggctggggtgccggcggcgggggcggcggcagtgactgcaccgggtggctgccgtgctcccgcgccaggcgctgcatgcgcgtgaagaccgccagggcgccggtgtagtcgcgcgccagcagctggcaggaggcggcctcgccaagcgcctgcagcgcggccaggggcagctggggcagctggagctgggcggcgcgctggaagtgaccggcggcggcggccggctggcccaggtcgcgcagggcggcggccagctcgaggcagagggcggcggcggcggccggctggcccagctcgaggtgcagacgcaccgcggcgcccagggcgctggcggcggcctgcagcggctccccgtaggcggcggggcagaccaggcgctggcgcgcgtcgcgctcctgccgcaggaagaggcgggcggcctcggtgagggccagcgcctccccgggcccgtggaagagcgcctgctggcagcgcgccaccgccagctggcaccaggccgcgtagggcagacactcctgggcgcgcagctcccggcccagctgtccgaactgctcgccggcctccgccacgttcggcttccgcaggaaccgcttcttcagcttgttcgataccagccggtagcgggccaggaagtccccggcctcgggtcccgggccggcgccgccgccgcccaggcctgcagccgctgccgccatgctcgccgccccaagcacttcccgacgcgccgccgcagctggcgggcgggccggggcggggcgacgtgccctgcgtccccctcggcgggctgccgccgtgcccgcgccggctccccagcccgagcctgccccttgccctgatgaggtgcaaagagcgggatcggaggcggggcctggccgggctgtgagcggcgtatgcaaatcgagggtctcggggatgcggatccaagaccctgggaaggtacgcggggcctggcggggcaccagctgctgctagctcggctgcaatgcaagtggtctaggttgctaaaggcatcccacagcctctccatctgaacatgacccaaacgaaactcgtgaccctaattccatgtctgcgcatttctagactgttgtccccccccccccccgccccgactactcagtcctccgtcttccggtccagggccccttgccaagcaccgggtccacctctccgtccccaccccggttgccttagaagtccgtcctgtcgcaacactgcagtcatggtcttgaggcccacccgccccaacgaacaccatcatgctgaggactttcccgggcaggccctgacttgctcagaaccagcgggggtgtccccttcccacccagggccactcccctgcactgtcacccggagagactgctcctctgtgccatccctggctcccacccaaccccagacccccaccacctctccatccctccagctgtggaggtctcacaaccccccaacccatctcaccgcccccccacccccaccccaaggcaaagtgactgaagcgggcagatggcttccttgaaacattttattgacagaattaatgaaggcccaagactttggggcctgggttgtggggggagggtgtttaaggccgggggttcaggccgggggatttggggccgggtgggtggacgagtggacctgtcaggtcccaggggccgggtgtcagaagctagtcctcgccaggggccacttgagagatggtggtcgtgttgaaaagggtgctcagtagcctgtcgttgtgaaccaccatgtccagcagcaggggagtgatgttccgctctccgctgttctgggcctcgttgcccgccagctccgggaccttggccgtcaggtactcaataaccgcagcgaggtagaccggcgccgtgcgactcaggcgctgagcgtagtggccctcccgtagactgcgctccacctggctcactgaaaacgaaagctccgctcggacggtgcgagagcaggtccgcccccggccgccagcaccggaggaccctcggcgtctcctcctcctcggcatgctgggcgttgagtgtgctatctcggcttggcccagctaggcaagatggctctcaagaggacagttaccgcgtccagtactgtgtatcctagcgaccagggcccagcccctcattggctagggagccgagaccaatgggcacgcacatccggcgacgggcacgcatgtggtgacggcccctcacaagggacacacgtccgtcaggtgacctcatcactttcccattggcctcgagggagcaggcctgggcctagaagtggctggagggccgtgggggtggggtggggcggggcagggggaatcgcgctggtgaccctctctttgccagtgggaactttccctttctactggatgggaacaccgtgggaaagacaaaggggtgggcgaggggaggacgggtaccacgccttcacaatgttgcacatccatcacgaccacctagttccaaaacgttttcaacaccccgaaaagaaaccgaaacccctgtacctataagcagtcacttgccgcacgcctccttccacaccaccactaccagcccccacaccctcccacacacaccccctgcccccgcccatacacacgttcccgatagtccctgacaacccctagtccatctgctttctgtccatagaggttagcctgttctggagatttcctatagatggaattatacgaccaaatgtgaggccgtgtgtgtctggctgctttcacttagcgtaatggtttcatcagggtgcatccatgtagaggcatgaatcactacttccttcctttgaatgactgagtacgattctgttgtatgaataggaggccacattttgtttacccactcgtcagttgatggacaggttatttcccccttctggctattgtgagtggcactgccatgaccatctctctacaggtttttctttgaatatctcttttcagttcttttgggtctatttctagcagtcaaactgctggctcgtgtggtaattctgtttaacttattgaggaaccaccaaactgatttccacagcagctgtaatctttcgcattcccaacagtagtgcatgagagtcccaatttcttcacagcctcatcaaaacctgttttctgtttgcctcattttgttttgtttacagtagccatcctactgggtgtcaagtgctatctcatggtggttttcattcgtatttcccaaatggctaatgatgttgctgtggtttgagtgcatcccccaaattgtgtgtcttggaaacttaatccccaaattcacatgttgattggaggcgcagcctctgagacggtaattaggattagataaggtcatcggggtgagacccccaggatgcgactggtggctttataagaataggaagagaggcctgaaacgacatacacgctcttgccctctcgccgtgtgataccctctgccgtccccagatgccgggtcacttcccagtccccagaacggtaagaaataaatttcttttctttataaattgttcagtgtcgggtattcaattatggcaacagaaaacagactaagacatcttttcatgtgcttcttggccctctgtacctctgctttggaggaatgtctattcaagccctttgcccattttttaattcggttgattgtattttggctgtgggcttctaaaacttattcatatattctggaaaatagactcttatcagatatgtgacttgcaaatgtttctcccattcactttctggatagagccctttgttgcccaaaagatttacatttggatgtagtccaacttgccaaatgaaaagatatctgtggctttgcctttggtgtcatactgaaggagctgttgcctaatccaaggtcgtgcaaagttacatctccgttttcttcttagagttttatagtttcagcccttacatttagatctgtgatccattttgaattaattctttacatgatgtgaggtaggggtccaggggccttcttttgcatgtggctatccagttgtcccagcgcagtttgttgaggggattattcttcccctccacccattgaggggtgccggaactcttactgaaaataaactttacataaatatatgggtttattcctgactctgagttctgtaacattgacctaatgtatcgatcacgatggcagtaccacccttttcggattactgcggttttgtagtacgttttgaaattgggaagtgtgagtccttcaacttttttcttttctgagattgttttggctatctgagccccttacattttcttatgaattttaggatcagcttgtcagtttttacaaagaaggcaggttggattctgacaggcatcacgatgaatctgtatattgccttggagattatgggcatcttaacaatattaagtgtcccaatccgttaacacaaaatgcctttcgatttatttaggtcttctttaatttattttagcaacgtcttgaaattttcagagtatacatcttgtacacctttagttaaatttattcctcgacattttattgtttcgatgctactgtaaaatgaatcatttccttaatcttattttcatgttattcattgctagggtgtagaaatacaaccgactgttgcagattgatcttggatactgcaactttgctgagccgaatatgctttgctgagcatactcagacagggttggcatattagtccgttcctacactgctataaagaactgcctgagaatgggtaattcctaaagaaaagaggtttaattgcctcatggttctgcaggctgtacaaggcttctgcttctgggcaggcctcaggaaacgtgcaatcatggcggaaggcgaaggggaagcaagcaccttcttcacatgttggagcaggaggaagagagagagaacgcacgcaaagggggaagcgctgcacattttcaaacaatcatcagatcttgtgagcgctctatcagaagaatagcaagggggaagtccgcccccatgattcaatcacctcccactaggcccttccttcaacaggtggggattacaattcgacatgagatttgggtggggacacagagccaaaccgtctcagtttttttttttttcttttgttggactctttagtgtcctctatataagaacatgccatctatgcatctatgaatagagatggttttacttgttcctttccgatctggatgccttttatttctttttcttgactaattgccctgactagaactttgagtacgatgttgagttacaagtggcattcctgatcttagggggaaatcaaccagtctttcaccattaagtatgatattatctctgggtttttcatggatgccctctatcaggttgaagaagtttctttctgttcctggtttgttgaatttattttcatgaaagggtactgcgttttgtcaaatgatcctttttgtacatgattaagatgaccatgagccccctcccccgcccccgctccgccatgcattctgttaatatggtgtattatataaattgattttcacatgttgaaccaaccttacatttgtgggataaatcctatttggtcatagtgtataaagagtggtcaataaacatttcgttgaaagaataggagtggatctggcaagcttcttggaggacaatgtgtgtgttaaagaatctgtagcatgatgagaagccaaggcaccggtgggaggaggggagttgcaaccaattcattaaggctggagagtacgatgccagtggagcagtagtggttgatgtggctgggaaagaggtaggcaggagccaagacatggaggttctattatgccatgctcaggttttagaataccctgtaggctacactgaacccactgtggtctttcagcttgggagtgacgtggtctgatttgcctctagaaatatcaccctggaagctgtgtggagaatagaacagagaggattgtgtgtggagaatagaacagagaggactgagattggaattagaaagctgctgtattataccagtcaagaaatgacagatatctcaactaagacaatggcattggtagataagactaggggacagagtccataaaaagtttaggtagtaaaatggcacacagtagacactcactacatattactcatactggcgaacctagctggagacatgataattcatgtgctcattcttcaaaaaatattgaagggtagtgccaggtatactgtgttaagcattgagacaacaccaacgagaaatat

SEQ ID NO: 4 - DNA, 13008 bp, Canis lupus familiaris
aagattttatttttatttatttgaaagagagcatgaggggatccctgggtggctcagcggtttagcgcctgcctttggcccagggcgtgatcctggagacccgggatcgagtcccacatcaggctccttgcatggagcttgcttctccctctgcctgtgtctccacctctctctgtgtgtttctcatgaataaataaataaattttcaaaagagagagagagcatgagtaagagggagagggagagatagagaatctaaagcagactctgtgctgagcaggaacccaacacagggctcaatcccacgaccctgagatcgtgacctgagccaaaaacaagagtcagatgcttaaccaactgagccacccaggcgcccctggagttgttttctaactcattaatttctgttcaaaactttaaaattttcttttactttctttcggttttgtctttcctaaaacatggagttgaatgactagttcatttattttcagtctttctcattcagtatgataaaagagttaactactctcatgaaggtcattcatttaataaacagttactgagtaactgctatgttctagattctagtacagagatggggaagctagagcccatccttgaatttggactaccacttgcttttgtacggactgtgacttaagaatggtttttacaggtttaaagttgcaaaaacaaacattatgcaacgaagatcatttgtggcctgaaaagactaaaatattgccatctggtcctttacagaaagtttgcagactgctggtctggcctaaaggcagtagagatgcctaggcagtgccatgaagcaggactcttcatccccacagcttgcctaatgtgcagatttcaatcttagtcatcgtcccccagtgtagtgattctcagatgtttttatatctttgttttgctcacagacaaaatcttgttcatcagagatatttcttatcatggatgtcccacataaagagggagaggggaacctttaaggaccacagctacactgccaccgttctcaatagtgtagaataatgtaaatgttaacttttttatttttttaagatttatttattcacgaaagacacagagagagaggcacagacagaggcagagggagaagcaggctccatgcagggagcccgacatgggactccatcctggggccccagcatcacgccctggactaaaggcggcgctaaaccgctgagccacctgggctgccctaacttttttattttttaaaagattttacttatttatccatgagagacacagagaggcagagacacaggcagagggaggagcaggcttcatgcagtgagcccgatgcgggactcgatcccaggaccccaggatcatgacctgagccaaaggcagatgctcagccactgagccacccaggtgcccctgtatatgttaactttgatatatcaatgaacatttcagtgatgtggctttttctctctggttttcaagttaaaaagaagagtatttttaatgtcctttaaaaatatttatttttggttgtgttagaaatcagtgttattttgacataaagttgataattaccaagggatttgtcaaagcctatgaaaattgcagaaatctagccttagcccagctatctatgctttgaagtttctgagggagagctataaaggagccaatgacaaatggaaaacaactttcatgttttctaaaattatacttgtatacccaacaccaggctctctggcaaaccctcccctctacatcctcaatgcaaggagttagaccagaggtccaagggtgcttttccttaagcccaaacccaaatactgccaccagtcacatatcaaaactcctatacattgttgttgtagtgatgtgatttgaagtgaggtttgggagccaatggcgaagaattcttgagactttttcagtgcaaaaaatgctgttttaattacagcacagggacaggacccatgggcagaaagacctgcactggggttgcgaggagtggctgattatgtaagattttccatcctatggaggggagggtgatgttaaggtcccaggaaattgagtatagggttcgggaggtctggctattgatgattgctttttttccttgtaaatcattaagacagttgcaaactgatggaagattcatgtcgtgcatgactgtgatctctgtcagttaagcatttgtttttccccttcctttgctcttgggcagccaggagtgcctgcacaacatcacacctttcccacctggtgggtggggtgggaggggggcagttgttgcggagtattagcgtgtgctttaccctcagcttgccttttgctccctcatcaataagactactggccagactgaggggggcacttgacgggatgagcactgggtgttactctagatgttggcaaattgaacaccaataaaaaataaatgtataaaaaaaaaaaagactactggccaggcctgtagcccgggttgagagtataccaagaaaagtaaaactgcaaaggaccatgcaccctaaccacttttttaaaaaatgtttttcaaaaattccagtataattaatgtagtgttacattagtttcaggtgtacaacatggtgactcaacacctctatacatttcccagggctcatgatgattacgtgcactcttaatccccatcatgtatttcacccatccccacacctacaccccatctggtgaccatcagtttctggtctatatttaggagtctggtttttttatctcttttttttctttcatcttttgtttcttaaattccacaggagtgaaatcatacagtatttgtctttctctgacttatttcacataacattatacattctagatccatccatgttgcaaatggcaagattgaattctttttcagggctcaaaaatactccattttggatctgtgtgtgtgtgtgtgtgtgtgtgtgtgtgtgtgtgtgtgtcttgatcctttcatctatggacacttggattgcttccatatattgactgttgtaaataatgctgctgtaaacataggggtgtgtatctttcttcgaattagtgttctcattttcgttgggtaaatacccagttggggaattacatggtcatatggtggttctatttttaatttttaaaggaacctccatactattttccacagtggccgcaacagctggcattcacaccaatagtgcatgaaggctcctttttctccacatcctcaccaacacctgtgctttcctgtggttttgattttagccattctgacagatgtgatatctcattgtggttttcacttgcatttccctgatgattagtgatgttgagcatcttttcatgtgtctgataccctaacacttttgcaataagttagactaggcttttagggctccgaaagacccttccaggcagccacgtgagtgcgcaggactggtggcggagtctgtgtcagatgggcctcttttgtattttcttacctactgactgcttccccgttgctgaaatggcggcatgaggactacctaaccgtcccacccatttacaggcgcttaactcacggtgaccaccgcctacacatcccccaacacacacacacactaaaggcaaaacagaactgcccaaccgcatccttaaacctcaccccaccagatcagttccgtacacagcctcaggctaaagggtgcattttccgaaagcagaaggactgagagggagattacattctggagagttctcactggccctcccaaacccctaaaggcaagtggaatgtaaaaacacgcggctagtaacgtttgcacgcgacatttggaccaaaaagccttgaaaatgtaggattctgaaacaggatgctgtcctcttgggcaagaaaggcgcggtctcgcagaccgaggaccacgcaataggtcggaagcacgctgattcaacacatctgagttacctaccagtggcgggaaggcgcccaggacaagtaagtcccagcgtggcccaggcccacgtctgagaatggaacctaggcccacaaccctgagttccaaggcacgccagacacctcgacagtcgaacgtgggcccctgctttgcgcaggacacattcgccttggcgccgaggaaggcccacgcggccaaggttgtctgtggattgactgtgcggcacagcccgagcagcaggcgcacggaccgctgcgagtgaacgaccacactgcggcccgaagcacagccacccgctcttccccttgctgcctcccgacaggtggagcagctattccgcgttacggaggaaggcgaaccgcaggcgagaggcatcagaacggctttattgtggatttagggcagcagccccgagggcccgtgccatctagtgctccccaggggtacgcgtggggcgtgggcaacaaaggagaacctgggtgagcacctggagagacaccggcctgcgctaaagcagatccccgacgaacaaaaaacggaaccgagaggcgtgtgcaacatccaaccgtccgacttgcaacagaggtgtacgggagggtgggggtgggggtgggggtgggggcccgcaggggagttgggtgcaagaagaggccaggggtaaaggggccgctcggtgtcccgtggcccgtcttggggaagagagccaagtcctccaggctgaccccgtgatgctggggtggttgccgcgccagggacggcacgaagcctgtgggatgcgggaggctgcagtcccgcagcgtccggtggaggcgggcgggcgaagagcaagacaggtgcgagtgccgggcccctgcccgtcggtccgtgggcaccgccgcccgccggccggccggccggccggccggccggcccgcggtccaacggcggggcagcagcaggccacggggccagaggcggaaagcggcttcggggctggcgcgcgcgagtggtcagacgccctgccccgacggggacacggcttcctgcagaacgaggtgcagcaggtggttctgctccgcactgagcagcggccacatgtccacctgcagcgacttgacggcctccgtgtccttctcgtgggtggccatgaccagggactggagcagcaggaacagctcgtcgggaagctggccggcgccgtcgggcccgtggccgtcgaaggcctcccaggagtacttctccagcgtgtgggcgtgctcgggcagcagcttggcgggcggcggctgcagcaggagcagcagcagcacgcgggacacctcgcagcggaccagcacgtccgagaaggcgcccagcgtggcgggcgcgggcgtgggcgtgggcgcgggcgcggcaggcagcagggcggcgggcagggccggggcggcggcggcggggcccagcggggcggaggccgacgaggacgaggccgaggccgacgaggtcgaggccgaggccgacgaggtcgacgccgccgccggcggggccaggggcagcggcggggcgggcggcggcggggccgggggcggctgccgcagcgggtggctgccgtgctcccgcgccaggcgctgcatgcgcgtgaagacggccagggcgccgctgtagtcgcgcgccagcagctggcaggaggcggcgtcgcccagcgcctgcagcgcggccaggggcagctgcggcaggtgcagctgcgcggcgcgcaggaagtggccggcggcggcggccggctggcccaggtcgcgcagggcggcggccagctcgaggcacaggccggcggcggcggccggctggcccagctccaggtgcaggcgcacggcggcgcccagcgcgctggcggcggcctgcagcggctccccgtaggccgcggggcaggcgaggcgctggcgggcgtcgcgctcctgccgcaggaagaggcgcgcggcctcggtcagcgccagcgcctccccgggcccgtggaacagcgcctgctggcagcgcgccacggccagctggcaccacgcggcgtacggcaggcactcctgcgcgcgcagctcccggcccagctgcgcgaactgctcgcccgcctccgccacgttcggcttccgcaggaaccgcttacgcagcttgctcgacacctgccggtagcgggccaggaagtccccggcctcgggccccgggcccgcgccgccgccgccgccgccgccgccgccgcccgggccgccgccgccgccgccgcccgggccgcccgccgccgccgccgccatcttgcccgcacgcgcgcacgcccgacgtgcccgcgtcccccggccccgccccctgcgggccccgcccccccgcggaccccgcgcatgcgtgcgccgccccccgccgtcccgccggacggaaccgagcgcgcgggccggcgcggggcctgggcggccgcggcccttccgaggcgaccccggcccccgggtcggcccgcgccccccggcccctcccggcccctgccggcccccgagctaacgtcgcggcgccggcccgcctggccccgaggccgcttggccggagtcaggatggtccccgcccccccagccttccgtcaaagccctgtcccctcgagtccgcgccggcacctgtgtcccccaacagtccgcgccggcagctgtgtccccccattcactccgcgccggcaggtgtgtccccctccatcccgcagccaggttgttactgcaccggcgttcaccccatcaccacgccgcaggcatggtcctgagctccagccccacacacaccatcgtccacgggactggcccgtgcggtgggggggggtcttctatgccccagcgtcactcccagcccagccaccccctgtcctgaccccgagcagtccccgtccccgcaccccagccggaccccaccaccacccctgcaccccagccggaccccgccacagcccccgtccctgcaccccaacaatgctccggaccgcatgaccgaaccccgcaccacacccacgaacccgcgccccacgccacaccccaaatcctccatcacccccatcgtgcaccgccgagggcaccccaaccccccgtcatccccgagccccgcacccccaccccaacctcgcccacaaccccaaaccccaacctcccccccgcccccccccgccctccccccgaggcgcgtcccgcacccagtgagccaggcgcacacgtctggttgtctctgcgccttttattgcggggacgcgggggtcaccgagcccccccggcggctccccgggcggcggcgggcatcaggggccgggggcggctagtaccgggccggggccacctgggacacggtggtcatcgtgaacaagccgctgagcagctcgtggttgtgcagcgcccggtccacgagctccggggtgatgtacgcggtgcgcctgtgccgggcctcgtcgcccgccagccccagcacggtggccgtcaggaactggatgacggccgccaggaagatgggggcggacgcgcccaggcgcttggcgtagcggccggcccgcaggaggcgctccatctggcacacggagaaggccagccccgcgcgggcgctgcgcgagcggcacgacctcgggcggccggcccgccctccacggctccccctgagccgcgcgcggggcctcggcggcgctcggcgcggggcctcgggctgcggcccggctgcggcccggctggggacgctcgggcgtcgggccgcggagccacgggcctcgggctgcggagaccccgggctgcggacgctcgggcgtcgggccgcggagccacgggcctcgggctgcggagaccccgggctgcggacggtcgggcgtcgggccgcggggacatggggcttgggctgcagagacatcgggctgcggacagagagacaccggcctcgggctgcggagagacggggcaagggctgcagacagacgggcctcaggctgcagagagaccgacctcgggctgcagagagaccgaactcgggctgcagagtgtctgacctcgggctgcagagaccgacctcgggctgcggagagacgggcctcgggctgcagaaagtccgacctcgggctgcagagaccgacctcaggctgcggagagacgggcctcgcgctgcagagagaccgacctcgggctgtagagagactgacctcgggctgcagagaccgacctcgggctgcagagagtccgacctcgggctgcagagagtccgacctcgggctgcagagagacgggcctcgggctgcgctgccgaaacagcgtcggggcgcagagaggagcgccggggtgcaccgccgtgcggcgcgctgggccggctgcacccgagccctcagcagcgggcgaggaggccccgctccgtatccgagggacacaccccctccccgccccgctgcgcacgcggtgacacgcaggcctgatgaggtcaccgcgtccccattggcccggcccggccctcgcccgccagaaaagccgctggcgggaagtcgctggctctgcgccgcgcggacggcatggggcgccaccgacgagcgtgcaggagctcgcgcgcccccacgtgcacccccgacatgtcggccctctcggctgcacacgcggcaccgccccgcacagacggcccggccgccgcgcgctcactgccccctgcaccccgtcctgcccccggggaccgaccgctcctcggcctcctgtccctgccgcttggcgtccgctggacacctgctgcaggggccaccctgggaccagtaggtggccgtgtgcgccggccgcgttccctcggcaccgtgttctcaggagggctgttctctgagggagcgggaaccggggtccctccccccgagagagcaggaatcgggcccctccccctgagggagcaggaatcggggcacccccccccagggagcaggaataacggcctcttccccccccccagggagcaggaatcggggcccctcccctcaagggagcaggagtcggggtccctcccccccgagagagcaggaatcgggcccctccccctgagggagcaggaatcggggtccctcctcccgagggagcaggaatcggggcacccccccccccagggagcaggaataacggcctcttcccccccccccccccgggagcaggaatcggggcccctcccctcgagggagcaggaatccgggacccccaagggagcgggaattggggtccctccgcccgagggagcaaaagacggacctcgggctgcagaaagacggacctcgggctgcggagagaccgacctcgggctgcggagagaccaacctcgggctgcgcttccgaaagacggcgtcggggcgcagagaggagcgccggggtgcaccgccgtgcggcgcgctgggccggctgctcccgagctctgagcagcgggcgaggaggccccgctccgtataaaagcgacaccccctcccctccccgctgcgcacgcggtgacacgcagatctgatgaggtcaccgcgtcctcattggcccggccctcgcccgccagaaaaggcgggaagtcgctggctctgcgccgcgcggacggcatggggcgccacccacgagcgtgcaggagctcgcgcgcccccacgtgcacccccgacatgtcggccctctcggctgcacacgcggcagcgccccgcacagacggcccggccgccgcgcgctcactgccccctgcaccccgtcctgcccccggggaccgaccgctcctcggcctcctgtccctgccgcttggcgtccgctggacacctgctgcaggggccaccctgggaccagtaggtggccgtgtgcgccggccgcgttccctcggcaccgtgttctcaggagggctgttctccgagggagcgggaacccgggtccccccccccaagggagcaggaattggggtccctccccccgagcgatcaggaagcggggtccctccaccaagggacaggagtcggggtccctccccccgagggatcaggaatcggggtccctccaccaagggatcaggagttggggtccctcccccaagggacaggagtcagggtccctcccccaagggacaggagtcggggtccctccgccaagggacaggagtcggggtccgtccccccgagggagcaggaataggccccccgaggcagcggggatcgccctgcacgtccatcgaggggcactcgcccccactgcgcgccccccctggcggcgaggggcacctgcgggcggacgtgcgcggcggcggcggcggcgaaggtcgcgcggggcccctccgggcgcgggatggggggcccgacggcagggcgacacccgctgtctgggcagcgcgctgacccggccccctgctcccgccgcgccgccccactggccctggcccgcgcctgctcctcccggtgcggcctcgcgagcccccgcgccggctgtgccgcggcacctggcacctgggggtcactgtcccccgtgtgtagggaggggcagggcggggcccgagggacagggagctcgggcagctgcagcccgctgacccgggcccccgtggagcctgcgggctccccccgcgcccccagggctgccgacccgagcccgggctgcaggcgggcgcccagctgatcccccccgccccccccccccccgggctgggcctgtcgcgcccccgggtcccgagcgccgccccgcggtgccagcagcggcgggtcggcgcggcgggagcgctgcaggtgcgccgggaccgggcggggccctccctctgggtgcccctccaggcggcccctgcactcgggctgcgcagggcggggcgggggagcttcccggagggggtgcggcctgtctgtcgcctgggcgcgactcggcgatgggacacgttcaggtcctgacaccgggggggggggggggagcgggggggcttcccgcgtattcggggcctcccgagtgactttcagcaatgttccgtgactttccgtgcacacgccctgcacgtcctccgctacgtgtattcctagggatgtaattgcacgtgatcccgatttgaataaaattattcaatcagttagttaactgatcaattaatcagtttcgtttgaggttcgtcgccgctgccgcgtggaaaaccccctaatttctgcacgttggtctcatatcctgaagtttgttgaattcactaactctgccggtgtttcgtgaattctttaggactttttctgtgtaaggttatgtcatctgagaacacagatggttttccttcttcctttccaatttaaataccctttatttctttctcttgcatcattgctctagccaggatttccattacaatgtcggttagaggcagggaaagcgcggattcttgttcctgattaggggaaaagctttcagtcctccaccagtgagtatgaccttagctatgggtatttcataaatgccctttattatgtttggtgattccccttctattcctagtttgctgagtgttttttgtcaggaaaaggtggattttagtcaatgctttttctgcatgaatcaagacagtcatgtgggtttttccccctttattttattaacgtagagttattttcttaagttgaagcatctttgtattcctgggacagttcctttttggacatgaaatgtcacttttataatgtactgctggattccgtctgctaaaatcatttgaggatttctgcacctatattcttttttaaagattttttaggtactatttgagagaccatgaatgatcagggggcggagggagaggatgaagcagactccccactgagcagggagcctgacgcgggcctcgatctcccgacccgggatcatgacctgagctgaaagcggatgcttcaccgactgagccaccaggcacccgggcaaaacaatttcttacaacattctgcacgatactgtaatgctgatgtgtcatcatataacacacactgattcctattctagtgtattcaagcatacacaaagcctaggagatcattttaaactttccgtagcctgtacgccatggtttaaaccgaggccttctgagtaggtgttccttttttatttaaagattttatttatttattcatgagagacacagagagagagagagaggcagagacccaggcagagggagaagcaggctccatgcagggagcccgacgcggggctcgatcccaggtctccaggttcatgccctgggccgaaggcaggtgccaagccactgagccccccagggatcccctgactaggtgttcctatcacatttctcaaactgtgttccctttcctttgaagatgccgtgtactttctctgcaccctagactgctcaaggtccgaacccccacatgttggatgttaacacgtgtcttacaaatccatacacaaggaatcattaattaaagcctcacagttcatgcacatgtgcacacacacacacacacagagagagaccacagtcttggaagattatcctgaggccagggtggtagggtggtgcctgccagcaccctctcagatgtggaacagggcccgacatacaggacttctagctacgacggttgtatgtgagcgctgcgtgctgtcgagagaagcacaaagcaaaattagagggaagatgcaatggggagcaattgctttgtaccctgtctgcacctggcatgtacctgtgctaatccctccccacaggtcttctttggcaacgtggattcatctgggatcaaacacaatatttttaaccctccgattattgctcagtacatccgtttgcacccaacccattacagcatccgcagcactcttcgcatggagctcttgggctgtgacttcaacagtaagtgcccagtcatcacgtgcccttccgtgtcccagccccgggtgggatgaatgactgtcctagtcttctcgagggcagggcgatgtcccaggacacagaaccacgaatgctaagagcagcgcagtcccgagcaaacgcaggccttggtcattgtaaccatgggattccctaggggcagccacctcctccggcactcttaaggtcaaagtgcccccgaactgagaagagctgaccagaaggcgcggggcag

SEQ ID NO: 5 - DNA, 1116 bp, Homo sapiens
atggcggcagcggctgcaggcctgggcggcggcggcgccggcccgggacccgaggccggggacttcctggcccgctaccggctggtatcgaacaagctgaagaagcggttcctgcggaagccgaacgtggcggaggccggcgagcagttcggacagctgggccgggagctgcgcgcccaggagtgtctgccctacgcggcctggtgccagctggcggtggcgcgctgccagcaggcgctcttccacgggcccggggaggcgctggccctcaccgaggccgcccgcctcttcctgcggcaggagcgcgacgcgcgccagcgcctggtctgccccgccgcctacggggagccgctgcaggccgccgccagcgccctgggcgccgcggtgcgtctgcacctcgagctgggccagccggccgccgccgccgccctctgcctcgagctggccgccgccctgcgcgacctgggccagccggccgccgccgccggtcacttccagcgcgccgcccagctccagctgccccagctgcccctggccgcgctgcaggcgcttggcgaggccgcctcctgccagctgctggcgcgcgactacaccggcgccctggcggtcttcacgcgcatgcagcgcctggcgcgggagcacggcagccacccggtgcagtcactgccgccgcccccgccgccggcaccccagcccgggcccggggcgacgcccgccctaccggccgcgctgcttcctccgaactccggctcggcggcgccctctcccgccgccctgggcgccttctcggacgtgctggtccgctgcgaggtgtcccgcgtgctgctgctgctcctcctgcaaccaccgcccgccaagctgctgccggagcacgcccagaccctggagaagtactcctgggaggcttttgacagccacgggcaggagagcagcggccagcttcccgaggagctctttctgctgctccagtctttggtcatggctacccacgaaaaggacacggaagccatcaagtcgctgcaggtggagatgtggccactgttgactgctgagcagaaccacctccttcacctcgttctgcaagaaaccatctccccctcaggacagggagtctga

SEQ ID NO: 6 - DNA, 1349 bp, Canis lupus familiaris
atgcgcggggtccgcgggggggcggggcccgcagggggcggggccgggggacgcgggcacgtcgggcgtgcgcgcgtgcgggcaagatggcggcggcggcggcgggcggcccgggcggcggcggcggcggcggcccgggcggcggcggcggcggcggcggcggcggcgcgggcccggggcccgaggccggggacttcctggcccgctaccggcaggtgtcgagcaagctgcgtaagcggttcctgcggaagccgaacgtggcggaggcgggcgagcagttcgcgcagctgggccgggagctgcgcgcgcaggagtgcctgccgtacgccgcgtggtgccagctggccgtggcgcgctgccagcaggcgctgttccacgggcccggggaggcgctggcgctgaccgaggccgcgcgcctcttcctgcggcaggagcgcgacgcccgccagcgcctcgcctgccccgcggcctacggggagccgctgcaggccgccgccagcgcgctgggcgccgccgtgcgcctgcacctggagctgggccagccggccgccgccgccggcctgtgcctcgagctggccgccgccctgcgcgacctgggccagccggccgccgccgccggccacttcctgcgcgccgcgcagctgcacctgccgcagctgcccctggccgcgctgcaggcgctgggcgacgccgcctcctgccagctgctggcgcgcgactacagcggcgccctggccgtcttcacgcgcatgcagcgcctggcgcgggagcacggcagccacccgctgcggcagccgcccccggccccgccgccgcccgccccgccgctgcccctggccccgccggcggcggcgtcgacctcgtcggcctcggcctcgacctcgtcggcctcggcctcgtcctcgtcggcctccgccccgctgggccccgccgccgccgccccggccctgcccgccgccctgctgcctgccgcgcccgcgcccacgcccacgcccgcgcccgccacgctgggcgccttctcggacgtgctggtccgctgcgaggtgtcccgcgtgctgctgctgctcctgctgcagccgccgcccgccaagctgctgcccgagcacgcccacacgctggagaagtactcctgggaggccttcgacggccacgggcccgacggcgccggccagcttcccgacgagctgttcctgctgctccagtccctggtcatggccacccacgagaaggacacggaggccgtcaagtcgctgcaggtggacatgtggccgctgctcagtgcggagcagaaccacctgctgcacctcgttctgcaggaagccgtgtccccgtcggggcagggcgtctga

SEQ ID NO: 7 - DNA, 22 bp, Homo sapiens
  misc_feature (22)..(22): n = c or g
ctcccaggagtacttctccagn

SEQ ID NO: 8 - DNA, 22 bp, Homo sapiens
  misc_feature (22)..(22): n = c or g
gagggtcctcatgaagaggtcn

SEQ ID NO: 9 - DNA, 22 bp, Homo sapiens
ctcccaggagtacttctccagg

SEQ ID NO: 10 - DNA, 22 bp, Homo sapiens
gagggtcctcatgaagaggtcc

SEQ ID NO: 11 - DNA, 22 bp, Canis lupus familiaris
ctcccaggagtacttctccagc

SEQ ID NO: 12 - DNA, 22 bp, Canis lupus familiaris
gagggtcctcatgaagaggtcg

SEQ ID NO: 13 - protein, 354 aa, Artificial sequence
  Synthesized
MNTKYNKEFLLYLAGFVDGDGSIYASIKPHQSVKFKHELRLGFSVGQKTQRRWFLDKLVDEIGVGYVRDKGSVSEYLLSQIKPLHNFLTQLQPFLKLKQKQANLVLKIIEQLPSAKESPDKFLEVCTWVDQIAALNDSKTRKTTSETVRAVLDSLPGSVGGLSPSQASSAASSASSSPGSGISEALRAGAGSGTGYNKEFLLYLAGFVDADGSIYAAIQPEQSSKFKHTLRLCFDVSQKTQRRWFLDKLVDEIGVGYVRDAGSVSHYVLSEIKPLHNFLTQLQPFLKLKQKQANLVLKIIEQLPSAKESPDKFLEVCTWVDQIAALNDSKTRKTTSETVRAVLDSLSEKKKSSP

SEQ ID NO: 14 - protein, 354 aa, Artificial sequence
  Synthesized
MNTKYNKEFLLYLAGFVDGDGSIYASIKPRQDLKFKHELRLGFSVGQKTQRRWFLDKLVDEIGVGYVRDKGSVSEYLLSQIKPLHNFLTQLQPFLKLKQKQANLVLKIIEQLPSAKESPDKFLEVCTWVDQIAALNDSKTRKTTSETVRAVLDSLPGSVGGLSPSQASSAASSASSSPGSGISEALRAGAGSGTGYNKEFLLYLAGFVDSDGSIYACIEPQQRMKFKHALRLSFNVSQKTQRRWFLDKLVDEIGVGYVRDNGSVSHYSLSEIKPLHNFLTQLQPFLKLKQKQANLVLKIIEQLPSAKESPDKFLEVCTWVDQIAALNDSKTRKTTSETVRAVLDSLSEKKKSSP

SEQ ID NO: 15 - protein, 354 aa, Artificial sequence
  Synthesized
MNTKYNKEFLLYLAGFVDGDGSIYASIKPAQDSKFKHNLRLGFSVGQKTQRRWFLDKLVDEIGVGYVRDKGSVSEYLLSQIKPLHNFLTQLQPFLKLKQKQANLVLKIIEQLPSAKESPDKFLEVCTWVDQIAALNDSKTRKTTSETVRAVLDSLPGSVGGLSPSQASSAASSASSSPGSGISEALRAGAGSGTGYNKEFLLYLAGFVDADGSIYATIQPEQSGKFKHTLRLCFDVSQKTQRRWFLDKLVDEIGVGYVRDAGSVSHYVLSEIKPLHNFLTQLQPFLKLKQKQANLVLKIIEQLPSAKESPDKFLEVCTWVDQIAALNDSKTRKTTSETVRAVLDSLSEKKKSSP

SEQ ID NO: 16 - protein, 354 aa, Artificial sequence
  Synthesized
MNTKYNKEFLLYLAGFVDGDGSIYASIKPAQDSKFKHNLRLGFSVGQKTQRRWFLDKLVDEIGVGYVRDKGSVSEYLLSQIKPLHNFLTQLQPFLKLKQKQANLVLKIIEQLPSAKESPDKFLEVCTWVDQIAALNDSKTRKTTSETVRAVLDSLPGSVGGLSPSQASSAASSASSSPGSGISEALRAGAGSGTGYNKEFLLYLAGFVDADGSIYATIEPEQDVKFKHTLRLVFNVSQKTQRRWLLDKLVDEIGVGYVNDKGSVSSYTLSKIKPLHNFLTQLQPFLKLKQKQANLVLKIIEQLPSAKESPDKFLEVCTWVDQIAALNDSKTRKTTSETVRAVLDSLSEKKKSSP

SEQ ID NO: 17 - protein, 354 aa, Artificial sequence
  Synthesized
MNTKYNKEFLLYLAGFVDGDGSIYASIKPAQDSKFKHNLRLGFSVGQKTQRRWFLDKLVDEIGVGYVRDKGSVSEYLLSEIKPLHNFLTQLQPFLKLKQKQANLVLKIIEQLPSAKESPDKFLEVCTWVDQIAALNDSKTRKTTSETVRAVLDSLPGSVGGLSPSQASSAASSASSSPGSGISEALRAGAGSGTGYNKEFLLYLAGFVDSDGSIYASIEPNQSPKFKHYLRLAFNVSQKTQRRWFLDKLVDEIGVGYVRDQGSVSHYTLSQIKPLHNFLTQLQPFLKLKQKQANLVLKIIEQLPSAKESPDKFLEVCTWVDQIAALNDSKTRKTTSETVRAVLDSLSEKKKSSP

SEQ ID NO: 18 - protein, 354 aa, Artificial sequence
  Synthesized
MNTKYNKEFLLYLAGFVDGDGSIYASIKPAQDSKFKHNLRLGFSVGQKTQRRWFLDKLVDEIGVGYVRDKGSVSEYLLSQIKPLHNFLTQLQPFLKLKQKQANLVLKIIEQLPSAKESPDKFLEVCTWVDQIAALNDSKTRKTTSETVRAVLDSLPGSVGGLSPSQASSAASSASSSPGSGISEALRAGAGSGTGYNKEFLLYLAGFVDSDGSIYACIEPQQRVKFKHALRLSFNVSQKTQRRWFLDKLVDEIGVGYVRDNGSVSHYQLSEIKPLHNFLTQLQPFLKLKQKQANLVLKIIEQLPSAKESPDKFLEVCTWVDQIAALNDSKTRKTTSETVRAVLDSLSEKKKSSP

SEQ ID NO: 19 - protein, 354 aa, Artificial sequence
  Synthesized
MNTKYNKEFLLYLAGFVDGDGSIYASIKPHQDLKFKHELRLGFEVSQKTQRRWFLDKLVDEIGVGYVRDRGSVSEYLLSQIKPLHNFLTQLQPFLKLKQKQANLVLKIIEQLPSAKESPDKFLEVCTWVDQIAALNDSKTRKTTSETVRAVLDSLPGSVGGLSPSQASSAASSASSSPGSGISEALRAGAGSGTGYNKEFLLYLAGFVDADGSIYAAIQPDQEVKFKHVLRLCFDVSQKTQRRWFLDKLVDEIGVGYVRDASSVSHYVLSEIKPLHNFLTQLQPFLKLKQKQANLVLKIIEQLPSAKESPDKFLEVCTWVDQIAALNDSKTRKTTSETVRAVLDSLSEKKKSSP

SEQ ID NO: 20 - protein, 354 aa, Artificial sequence
  Synthesized
MNTKYNKEFLLYLAGFVDGDGSIYASIKPHQDLKFKHELRLGFEVSQKTQRRWFLDKLVDEIGVGYVRDRGSVSEYLLSQIKPLHNFLTQLQPFLKLKQKQANLVLKIIEQLPSAKESPDKFLEVCTWVDQIAALNDSKTRKTTSETVRAVLDSLPGSVGGLSPSQASSAASSASSSPGSGISEALRAGAGSGTGYNKEFLLYLAGFVDADGSIYAAIQPDQEVKFKHVLRLCFDVSQKTQRRWFLDKLVDEIGVGYVRDAGSVSHYVLSEIKPLHNFLTQLQPFLKLKQKQANLVLKIIEQLPSAKESPDKFLEVCTWVDQIAALNDSKTRKTTSETVRAVLDSLSEKKKSSP

SEQ ID NO: 21 - protein, 354 aa, Artificial sequence
  Synthesized
MNTKYNKEFLLYLAGFVDGDGSIYASIKPHQDLKFKHELRLGFEVGQKTQRRWFLDKLVDEIGVGYVRDRGSVSHYLLSQIKPLHNFLTQLQPFLKLKQKQANLVLKIIEQLPSAKESPDKFLEVCTWVDQIAALNDSKTRKTTSETVRAVLDSLPGSVGGLSSSQASSAASSASSSPGSGISEALRAGAGSGTGYNKEFLLYLAGFVDADGSIYAAIQPDQKVKFKHVLRLCFDVSQKTQRRWFLDKLVDEIGVGYVRDAYPCAHYVLSEIKPLHNFLTQLQPFLKLKQKQANLVLKIIEQLPSAKESPDKFLEVCTWVDQIAALNDSKTRKTTSETVRAVLDSLSEKKKSSP

SEQ ID NO: 22 - protein, 147 aa, Artificial sequence
  Synthesized
KEFLLYLAGFVDGDGSIYASIKPHQSVKFKHELRLGFSVGQKTQRRWFLDKLVDEIGVGYVRDKGSVSEYLLSQIKPLHNFLTQLQPFLKLKQKQANLVLKIIEQLPSAKESPDKFLEVCTWVDQIAALNDSKTRKTTSETVRAVLD

SEQ ID NO: 23 - protein, 147 aa, Artificial sequence
  Synthesized
KEFLLYLAGFVDGDGSIYASIKPRQDLKFKHELRLGFSVGQKTQRRWFLDKLVDEIGVGYVRDKGSVSEYLLSQIKPLHNFLTQLQPFLKLKQKQANLVLKIIEQLPSAKESPDKFLEVCTWVDQIAALNDSKTRKTTSETVRAVLD

SEQ ID NO: 24 - protein, 147 aa, Artificial sequence
  Synthesized
KEFLLYLAGFVDGDGSIYASIKPAQDSKFKHNLRLGFSVGQKTQRRWFLDKLVDEIGVGYVRDKGSVSEYLLSQIKPLHNFLTQLQPFLKLKQKQANLVLKIIEQLPSAKESPDKFLEVCTWVDQIAALNDSKTRKTTSETVRAVLD

SEQ ID NO: 25 - protein, 147 aa, Artificial sequence; identical to SEQ ID NO: 24
  Synthesized

SEQ ID NO: 26 - protein, 147 aa, Artificial sequence
  Synthesized
KEFLLYLAGFVDGDGSIYASIKPAQDSKFKHNLRLGFSVGQKTQRRWFLDKLVDEIGVGYVRDKGSVSEYLLSEIKPLHNFLTQLQPFLKLKQKQANLVLKIIEQLPSAKESPDKFLEVCTWVDQIAALNDSKTRKTTSETVRAVLD

SEQ ID NO: 27 - protein, 147 aa, Artificial sequence; identical to SEQ ID NO: 24
  Synthesized

SEQ ID NO: 28 - protein, 147 aa, Artificial sequence
  Synthesized
KEFLLYLAGFVDGDGSIYASIKPHQDLKFKHELRLGFEVSQKTQRRWFLDKLVDEIGVGYVRDRGSVSEYLLSQIKPLHNFLTQLQPFLKLKQKQANLVLKIIEQLPSAKESPDKFLEVCTWVDQIAALNDSKTRKTTSETVRAVLD

SEQ ID NO: 29 - protein, 147 aa, Artificial sequence; identical to SEQ ID NO: 28
  Synthesized

SEQ ID NO: 30 - protein, 147 aa, Artificial sequence
  Synthesized
KEFLLYLAGFVDGDGSIYASIKPHQDLKFKHELRLGFEVGQKTQRRWFLDKLVDEIGVGYVRDRGSVSHYLLSQIKPLHNFLTQLQPFLKLKQKQANLVLKIIEQLPSAKESPDKFLEVCTWVDQIAALNDSKTRKTTSETVRAVLD

SEQ ID NO: 31 - protein, 147 aa, Artificial sequence
  Synthesized
KEFLLYLAGFVDADGSIYAAIQPEQSSKFKHTLRLCFDVSQKTQRRWFLDKLVDEIGVGYVRDAGSVSHYVLSEIKPLHNFLTQLQPFLKLKQKQANLVLKIIEQLPSAKESPDKFLEVCTWVDQIAALNDSKTRKTTSETVRAVLD

SEQ ID NO: 32 - protein, 147 aa, Artificial sequence
  Synthesized
KEFLLYLAGFVDSDGSIYACIEPQQRMKFKHALRLSFNVSQKTQRRWFLDKLVDEIGVGYVRDNGSVSHYSLSEIKPLHNFLTQLQPFLKLKQKQANLVLKIIEQLPSAKESPDKFLEVCTWVDQIAALNDSKTRKTTSETVRAVLD

SEQ ID NO: 33 - protein, 147 aa, Artificial sequence
  Synthesized
KEFLLYLAGFVDADGSIYATIQPEQSGKFKHTLRLCFDVSQKTQRRWFLDKLVDEIGVGYVRDAGSVSHYVLSEIKPLHNFLTQLQPFLKLKQKQANLVLKIIEQLPSAKESPDKFLEVCTWVDQIAALNDSKTRKTTSETVRAVLD

SEQ ID NO: 34 - protein, 147 aa, Artificial sequence
  Synthesized
KEFLLYLAGFVDADGSIYATIEPEQDVKFKHTLRLVFNVSQKTQRRWLLDKLVDEIGVGYVNDKGSVSSYTLSKIKPLHNFLTQLQPFLKLKQKQANLVLKIIEQLPSAKESPDKFLEVCTWVDQIAALNDSKTRKTTSETVRAVLD

SEQ ID NO: 35 - protein, 147 aa, Artificial sequence
  Synthesized
KEFLLYLAGFVDSDGSIYASIEPNQSPKFKHYLRLAFNVSQKTQRRWFLDKLVDEIGVGYVRDQGSVSHYTLSQIKPLHNFLTQLQPFLKLKQKQANLVLKIIEQLPSAKESPDKFLEVCTWVDQIAALNDSKTRKTTSETVRAVLD

SEQ ID NO: 36 - protein, 147 aa, Artificial sequence
  Synthesized
KEFLLYLAGFVDSDGSIYACIEPQQRVKFKHALRLSFNVSQKTQRRWFLDKLVDEIGVGYVRDNGSVSHYQLSEIKPLHNFLTQLQPFLKLKQKQANLVLKIIEQLPSAKESPDKFLEVCTWVDQIAALNDSKTRKTTSETVRAVLD

SEQ ID NO: 37 - protein, 147 aa, Artificial sequence
  Synthesized
KEFLLYLAGFVDADGSIYAAIQPDQEVKFKHVLRLCFDVSQKTQRRWFLDKLVDEIGVGYVRDASSVSHYVLSEIKPLHNFLTQLQPFLKLKQKQANLVLKIIEQLPSAKESPDKFLEVCTWVDQIAALNDSKTRKTTSETVRAVLD

SEQ ID NO: 38 - protein, 147 aa, Artificial sequence
  Synthesized
KEFLLYLAGFVDADGSIYAAIQPDQEVKFKHVLRLCFDVSQKTQRRWFLDKLVDEIGVGYVRDAGSVSHYVLSEIKPLHNFLTQLQPFLKLKQKQANLVLKIIEQLPSAKESPDKFLEVCTWVDQIAALNDSKTRKTTSETVRAVLD

SEQ ID NO: 39 - protein, 147 aa, Artificial sequence
  Synthesized
KEFLLYLAGFVDADGSIYAAIQPDQKVKFKHVLRLCFDVSQKTQRRWFLDKLVDEIGVGYVRDAYPCAHYVLSEIKPLHNFLTQLQPFLKLKQKQANLVLKIIEQLPSAKESPDKFLEVCTWVDQIAALNDSKTRKTTSETVRAVLD

SEQ ID NO: 40 - DNA, 38 bp, Artificial sequence
  Synthesized
cccttacagttattaactactctcatgaggttcattcc

SEQ ID NO: 41 - DNA, 39 bp, Artificial sequence
  Synthesized
ggccctacaaccattctgcctttcactttcagtgcaata

SEQ ID NO: 42 - DNA, 36 bp, Artificial sequence
  Synthesized
cacaagggggaagagtgtgagggtgtgggataagaa

SEQ ID NO: 43 - DNA, 18 bp, Artificial sequence
  Synthesized
gagccagttgtgtaccat

SEQ ID NO: 44 - DNA, 20 bp, Artificial sequence
  Synthesized
acgtgatcccgatttgaata

SEQ ID NO: 45 - DNA, 18 bp, Artificial sequence
  Synthesized
gcaccttactgtcctgat

SEQ ID NO: 46 - DNA, 22 bp, Homo sapiens
ttcccagtagtacttctccagt

SEQ ID NO: 47 - DNA, 17 bp, Artificial sequence
  Synthesized
tctggatggcaacaagt

SEQ ID NO: 48 - DNA, 9 bp, Artificial sequence
  Synthesized
tgccaaaga

SEQ ID NO: 49 - DNA, 16 bp, Artificial sequence
  Synthesized
agaccattaaggtccc

SEQ ID NO: 50 - DNA, 19 bp, Artificial sequence
  Synthesized
tgatcccagatgaatccac